European Patent Application EP 4 495 143 A1, published January 22, 2025. Title: HUMAN INSULIN ANALOGUE, AND FUSION PROTEIN THEREOF AND MEDICAL USE THEREOF. Applicant: BEIJING TUOJIE BIOPHARMACEUTICAL CO., LTD. Application WO. The sequence listing filed with the application follows.

SEQUENCE LISTING (55 sequences)

SEQ ID NO: 1 - protein, 26 aa, synthetic construct
  source 1..26: note; note (original language) = Insulin B-chain analog
  VARIANT 3: note; note (original language) = X is selected from the group consisting of N, G, and K
  VARIANT 9: note; note (original language) = X is selected from the group consisting of S and E
  VARIANT 16: note; note (original language) = X is selected from the group consisting of Y, H, and E
  VARIANT 17: note; note (original language) = X is selected from the group consisting of H, R, L, and E
  VARIANT 25: note; note (original language) = X is selected from the group consisting of F and H
FVXQHLCGXHLVEALXXVCGERGFXY

SEQ ID NO: 2 - protein, 21 aa, synthetic construct
  source 1..21: note; note (original language) = Insulin A-chain analog
  VARIANT 8: note; note (original language) = Z is selected from the group consisting of T, H, and E
  VARIANT 14: note; note (original language) = Z is selected from the group consisting of Y, D, S, and E
  VARIANT 21: note; note (original language) = Z is selected from the group consisting of G and N
GIVEQCCZSICSLZQLENYCZ

SEQ ID NO: 3 - protein, 11 aa, synthetic construct
  source 1..11: note; note (original language) = Linker
GGGGGGSGGGG

SEQ ID NO: 4 - protein, 58 aa, synthetic construct
  source 1..58: note; note (original language) = Human insulin analog 1
FVNQHLCGEHLVEALYLVCGERGFHYGGGGGGSGGGGGIVEQCCESICSLEQLENYCG

SEQ ID NO: 5 - protein, 58 aa, synthetic construct
  source 1..58: note; note (original language) = Human insulin analog 2
FVNQHLCGSHLVEALYLVCGERGFHYGGGGGGSGGGGGIVEQCCHSICSLEQLENYCG

SEQ ID NO: 6 - protein, 58 aa, synthetic construct
  source 1..58: note; note (original language) = Human insulin analog 3
FVNQHLCGSHLVEALHLVCGERGFHYGGGGGGSGGGGGIVEQCCTSICSLEQLENYCN

SEQ ID NO: 7 - protein, 58 aa, synthetic construct
  source 1..58: note; note (original language) = Human insulin analog 4
FVKQHLCGEHLVEALYLVCGERGFHYGGGGGGSGGGGGIVEQCCESICSLEQLENYCG

SEQ ID NO: 8 - protein, 57 aa, synthetic construct
  source 1..57: note; note (original language) = Human insulin analog 5
FVNQHLCGEHLVEALYLVCGERGFHYGGGGGSGGGGGIVEQCCESICSLEQLENYCG

SEQ ID NO: 9 - protein, 58 aa, synthetic construct
  source 1..58: note; note (original language) = Human insulin analog 6
FVNQHLCGEHLVEALYLVCGERGFHYGGGGGGSGGGGGIVEQCCESICSLEQLENYCN

SEQ ID NO: 10 - protein, 20 aa, synthetic construct
  source 1..20: note; note (original language) = Linker sequence for fusion of human insulin analog with Fc
GGGGQGGGGQGGGGQGGGGG

SEQ ID NO: 11 - protein, 20 aa, synthetic construct
  source 1..20: note; note (original language) = Linker sequence for fusion of human insulin analog with Fc
HGGGQGGGGQGGGGQGGGGG

SEQ ID NO: 12 - protein, 25 aa, synthetic construct
  source 1..25: note; note (original language) = Linker sequence for fusion of human insulin analog with Fc
GGGGQGGGGQGGGGQGGGGQGGGGQ

SEQ ID NO: 13 - protein, 32 aa, synthetic construct
  source 1..32: note; note (original language) = Linker sequence for fusion of human insulin analog with Fc
PGPQPGPQPGPQPGPQPGPQPGPQPGPQPGPQ

SEQ ID NO: 14 - protein, 25 aa, synthetic construct
  source 1..25: note; note (original language) = Linker sequence for fusion of human insulin analog with Fc
GGGGQGGGGQGGGGQGGGGGQGGGG

SEQ ID NO: 15 - protein, 20 aa, synthetic construct
  source 1..20: note; note (original language) = Linker sequence for fusion of human insulin analog with Fc
GGGGAGGGGAGGGGAGGGGG

SEQ ID NO: 16 - protein, 34 aa, synthetic construct
  source 1..34: note; note (original language) = Linker sequence for fusion of human insulin analog with Fc
GGGGQGGGGQGGGGQGGGGQGGPCPPCPAPEAAG

SEQ ID NO: 17 - protein, 221 aa, Homo sapiens
  source 1..221: note = IgG2 Fc1
ECPPCPAPPVAGPSVFLFPPKPKDTLMISRTPEVTCVVVDVSHEDPEVQFNWYVDGVEVHNAKTKPREEQFNSTFRVVSVLTVVHQDWLNGKEYKCKVSNKGLPAPIEKTISKTKGQPREPQVYTLPPSREEMTKNQVSLTCLVKGFYPSDIAVEWESNGQPENNYKTTPPMLDSDGSFFLYSKLTVDKSRWQQGNVFSCSVMHEALHNHYTQKSLSLSPG

SEQ ID NO: 18 - protein, 210 aa, Homo sapiens
  source 1..210: note = IgG2 Fc2
GPSVFLFPPKPKDTLMISRTPEVTCVVVDVSHEDPEVQFNWYVDGVEVHNAKTKPREEQFNSTFRVVSVLTVVHQDWLNGKEYKCKVSNKGLPAPIEKTISKTKGQPREPQVYTLPPSREEMTKNQVSLTCLVKGFYPSDIAVEWESNGQPENNYKTTPPMLDSDGSFFLYSKLTVDKSRWQQGNVFSCSVMHEALHNHYTQKSLSLSPG

SEQ ID NO: 19 - protein, 299 aa, synthetic construct
  source 1..299: note; note (original language) = Fusion protein 1
FVNQHLCGEHLVEALYLVCGERGFHYGGGGGGSGGGGGIVEQCCESICSLEQLENYCGGGGGQGGGGQGGGGQGGGGGECPPCPAPPVAGPSVFLFPPKPKDTLMISRTPEVTCVVVDVSHEDPEVQFNWYVDGVEVHNAKTKPREEQFNSTFRVVSVLTVVHQDWLNGKEYKCKVSNKGLPAPIEKTISKTKGQPREPQVYTLPPSREEMTKNQVSLTCLVKGFYPSDIAVEWESNGQPENNYKTTPPMLDSDGSFFLYSKLTVDKSRWQQGNVFSCSVMHEALHNHYTQKSLSLSPG

SEQ ID NO: 20 - protein, 299 aa, synthetic construct
  source 1..299: note; note (original language) = Fusion protein 2
FVNQHLCGSHLVEALYLVCGERGFHYGGGGGGSGGGGGIVEQCCHSICSLEQLENYCGGGGGQGGGGQGGGGQGGGGGECPPCPAPPVAGPSVFLFPPKPKDTLMISRTPEVTCVVVDVSHEDPEVQFNWYVDGVEVHNAKTKPREEQFNSTFRVVSVLTVVHQDWLNGKEYKCKVSNKGLPAPIEKTISKTKGQPREPQVYTLPPSREEMTKNQVSLTCLVKGFYPSDIAVEWESNGQPENNYKTTPPMLDSDGSFFLYSKLTVDKSRWQQGNVFSCSVMHEALHNHYTQKSLSLSPG

SEQ ID NO: 21 - protein, 299 aa, synthetic construct
  source 1..299: note; note (original language) = Fusion protein 3
FVNQHLCGSHLVEALHLVCGERGFHYGGGGGGSGGGGGIVEQCCTSICSLEQLENYCNGGGGQGGGGQGGGGQGGGGGECPPCPAPPVAGPSVFLFPPKPKDTLMISRTPEVTCVVVDVSHEDPEVQFNWYVDGVEVHNAKTKPREEQFNSTFRVVSVLTVVHQDWLNGKEYKCKVSNKGLPAPIEKTISKTKGQPREPQVYTLPPSREEMTKNQVSLTCLVKGFYPSDIAVEWESNGQPENNYKTTPPMLDSDGSFFLYSKLTVDKSRWQQGNVFSCSVMHEALHNHYTQKSLSLSPG

SEQ ID NO: 22 - protein, 299 aa, synthetic construct
  source 1..299: note; note (original language) = Fusion protein 4
FVKQHLCGEHLVEALYLVCGERGFHYGGGGGGSGGGGGIVEQCCESICSLEQLENYCGGGGGQGGGGQGGGGQGGGGGECPPCPAPPVAGPSVFLFPPKPKDTLMISRTPEVTCVVVDVSHEDPEVQFNWYVDGVEVHNAKTKPREEQFNSTFRVVSVLTVVHQDWLNGKEYKCKVSNKGLPAPIEKTISKTKGQPREPQVYTLPPSREEMTKNQVSLTCLVKGFYPSDIAVEWESNGQPENNYKTTPPMLDSDGSFFLYSKLTVDKSRWQQGNVFSCSVMHEALHNHYTQKSLSLSPG

SEQ ID NO: 23 - protein, 304 aa, synthetic construct
  source 1..304: note; note (original language) = Fusion protein 5
FVNQHLCGEHLVEALYLVCGERGFHYGGGGGGSGGGGGIVEQCCESICSLEQLENYCGGGGGQGGGGQGGGGQGGGGQGGGGQECPPCPAPPVAGPSVFLFPPKPKDTLMISRTPEVTCVVVDVSHEDPEVQFNWYVDGVEVHNAKTKPREEQFNSTFRVVSVLTVVHQDWLNGKEYKCKVSNKGLPAPIEKTISKTKGQPREPQVYTLPPSREEMTKNQVSLTCLVKGFYPSDIAVEWESNGQPENNYKTTPPMLDSDGSFFLYSKLTVDKSRWQQGNVFSCSVMHEALHNHYTQKSLSLSPG

SEQ ID NO: 24 - protein, 298 aa, synthetic construct
  source 1..298: note; note (original language) = Fusion protein 6
FVNQHLCGEHLVEALYLVCGERGFHYGGGGGSGGGGGIVEQCCESICSLEQLENYCGGGGGQGGGGQGGGGQGGGGGECPPCPAPPVAGPSVFLFPPKPKDTLMISRTPEVTCVVVDVSHEDPEVQFNWYVDGVEVHNAKTKPREEQFNSTFRVVSVLTVVHQDWLNGKEYKCKVSNKGLPAPIEKTISKTKGQPREPQVYTLPPSREEMTKNQVSLTCLVKGFYPSDIAVEWESNGQPENNYKTTPPMLDSDGSFFLYSKLTVDKSRWQQGNVFSCSVMHEALHNHYTQKSLSLSPG

SEQ ID NO: 25 - protein, 311 aa, synthetic construct
  source 1..311: note; note (original language) = Fusion protein 7
FVNQHLCGEHLVEALYLVCGERGFHYGGGGGGSGGGGGIVEQCCESICSLEQLENYCGPGPQPGPQPGPQPGPQPGPQPGPQPGPQPGPQECPPCPAPPVAGPSVFLFPPKPKDTLMISRTPEVTCVVVDVSHEDPEVQFNWYVDGVEVHNAKTKPREEQFNSTFRVVSVLTVVHQDWLNGKEYKCKVSNKGLPAPIEKTISKTKGQPREPQVYTLPPSREEMTKNQVSLTCLVKGFYPSDIAVEWESNGQPENNYKTTPPMLDSDGSFFLYSKLTVDKSRWQQGNVFSCSVMHEALHNHYTQKSLSLSPG

SEQ ID NO: 26 - protein, 299 aa, synthetic construct
  source 1..299: note; note (original language) = Fusion protein 8
FVNQHLCGEHLVEALYLVCGERGFHYGGGGGGSGGGGGIVEQCCESICSLEQLENYCGGGGGAGGGGAGGGGAGGGGGECPPCPAPPVAGPSVFLFPPKPKDTLMISRTPEVTCVVVDVSHEDPEVQFNWYVDGVEVHNAKTKPREEQFNSTFRVVSVLTVVHQDWLNGKEYKCKVSNKGLPAPIEKTISKTKGQPREPQVYTLPPSREEMTKNQVSLTCLVKGFYPSDIAVEWESNGQPENNYKTTPPMLDSDGSFFLYSKLTVDKSRWQQGNVFSCSVMHEALHNHYTQKSLSLSPG

SEQ ID NO: 27 - protein, 299 aa, synthetic construct
  source 1..299: note; note (original language) = Fusion protein 9
FVNQHLCGEHLVEALYLVCGERGFHYGGGGGGSGGGGGIVEQCCESICSLEQLENYCNHGGGQGGGGQGGGGQGGGGGECPPCPAPPVAGPSVFLFPPKPKDTLMISRTPEVTCVVVDVSHEDPEVQFNWYVDGVEVHNAKTKPREEQFNSTFRVVSVLTVVHQDWLNGKEYKCKVSNKGLPAPIEKTISKTKGQPREPQVYTLPPSREEMTKNQVSLTCLVKGFYPSDIAVEWESNGQPENNYKTTPPMLDSDGSFFLYSKLTVDKSRWQQGNVFSCSVMHEALHNHYTQKSLSLSPG

SEQ ID NO: 28 - protein, 299 aa, synthetic construct
  source 1..299: note = LY3209590
FVNQHLCGSHLVEALELVCGERGFHYGGGGGGSGGGGGIVEQCCTSTCSLDQLENYCGGGGGQGGGGQGGGGQGGGGGECPPCPAPPVAGPSVFLFPPKPKDTLMISRTPEVTCVVVDVSHEDPEVQFNWYVDGVEVHNAKTKPREEQFNSTFRVVSVLTVVHQDWLNGKEYKCKVSNKGLPAPIEKTISKTKGQPREPQVYTLPPSREEMTKNQVSLTCLVKGFYPSDIAVEWESNGQPENNYKTTPPMLDSDGSFFLYSKLTVDKSRWQQGNVFSCSVMHEALHNHYTQKSLSLSPG

SEQ ID NO: 29 - protein, 21 aa, Homo sapiens
  source 1..21: note; note (original language) = A-chain
GIVEQCCTSICSLYQLENYCN

SEQ ID NO: 30 - protein, 30 aa, Homo sapiens
  source 1..30: note; note (original language) = B-chain
FVNQHLCGSHLVEALYLVCGERGFFYTPKT

SEQ ID NO: 31 - protein, 26 aa, synthetic construct
  source 1..26: note; note (original language) = Insulin B-chain analog
FVNQHLCGEHLVEALYLVCGERGFHY

SEQ ID NO: 32 - protein, 26 aa, synthetic construct
  source 1..26: note; note (original language) = Insulin B-chain analog
FVNQHLCGSHLVEALYLVCGERGFHY

SEQ ID NO: 33 - protein, 26 aa, synthetic construct
  source 1..26: note; note (original language) = Insulin B-chain analog
FVNQHLCGSHLVEALHLVCGERGFHY

SEQ ID NO: 34 - protein, 26 aa, synthetic construct
  source 1..26: note; note (original language) = Insulin B-chain analog
FVKQHLCGEHLVEALYLVCGERGFHY

SEQ ID NO: 35 - protein, 26 aa, synthetic construct
  source 1..26: note; note (original language) = Insulin B-chain analog
FVNQHLCGEHLVEALYLVCGERGFHY

SEQ ID NO: 36 - protein, 26 aa, synthetic construct
  source 1..26: note; note (original language) = Insulin B-chain analog
FVNQHLCGEHLVEALYLVCGERGFHY

SEQ ID NO: 37 - protein, 21 aa, synthetic construct
  source 1..21: note; note (original language) = Insulin A in insulin analog
GIVEQCCESICSLEQLENYCG

SEQ ID NO: 38 - protein, 21 aa, synthetic construct
  source 1..21: note; note (original language) = Insulin A in insulin analog
GIVEQCCHSICSLEQLENYCG

SEQ ID NO: 39 - protein, 21 aa, synthetic construct
  source 1..21: note; note (original language) = Insulin A in insulin analog
GIVEQCCTSICSLEQLENYCN

SEQ ID NO: 40 - protein, 21 aa, synthetic construct
  source 1..21: note; note (original language) = Insulin A in insulin analog
GIVEQCCESICSLEQLENYCG

SEQ ID NO: 41 - protein, 21 aa, synthetic construct
  source 1..21: note; note (original language) = Insulin A in insulin analog
GIVEQCCESICSLEQLENYCG

SEQ ID NO: 42 - protein, 21 aa, synthetic construct
  source 1..21: note; note (original language) = Insulin A in insulin analog
GIVEQCCESICSLEQLENYCN

SEQ ID NO: 43 - protein, 29 aa, synthetic construct
  source 1..29: note; note (original language) = Insulin B-chain analog
  VARIANT 3: note; note (original language) = X is selected from the group consisting of N, G, and K
  VARIANT 9: note; note (original language) = X is selected from the group consisting of S and E
  VARIANT 16: note; note (original language) = X is selected from the group consisting of Y, H, and E
  VARIANT 17: note; note (original language) = X is selected from the group consisting of H, R, L, and E
  VARIANT 25: note; note (original language) = X is selected from the group consisting of F and H
  VARIANT 26: note; note (original language) = X is selected from the group consisting of G, T, S, H, V, and Y, or is absent
  VARIANT 27: note; note (original language) = X is selected from the group consisting of G, E, P, K, D, S, and H, or is absent
  VARIANT 28: note; note (original language) = X is selected from the group consisting of G, E, K, P, Q, D, and H, or is absent
  VARIANT 29: note; note (original language) = X is selected from the group consisting of G, T, S, E, K, and A, or is absent
FVXQHLCGXHLVEALXXVCGERGFXXXXX

SEQ ID NO: 44 - protein, 22 aa, synthetic construct
  source 1..22: note; note (original language) = Insulin A-chain analog
  VARIANT 8: note; note (original language) = Z is selected from the group consisting of T, H, and E
  VARIANT 14: note; note (original language) = Z is selected from the group consisting of Y, D, S, and E
  VARIANT 21: note; note (original language) = Z is selected from the group consisting of G and N
  VARIANT 22: note; note (original language) = Z is any natural amino acid or is absent
GIVEQCCZSICSLZQLENYCZZ

SEQ ID NO: 45 - protein, 7 aa, synthetic construct
  source 1..7: note; note (original language) = Linker
GGSGGGG

SEQ ID NO: 46 - protein, 6 aa, synthetic construct
  source 1..6: note; note (original language) = Linker
GSGGGG

SEQ ID NO: 47 - protein, 5 aa, synthetic construct
  source 1..5: note; note (original language) = Linker
GGGGG

SEQ ID NO: 48 - protein, 232 aa, Homo sapiens
  source 1..232: note; note (original language) = Human IgG1 Fc region 1
EPKSCDKTHTCPPCPAPEAAGGPSVFLFPPKPKDTLMISRTPEVTCVVVDVSHEDPEVKFNWYVDGVEVHNAKTKPREEQYNSTYRVVSVLTVLHQDWLNGKEYKCKVSNKALPAPIEKTISKAKGQPREPQVYTLPPSREEMTKNQVSLTCLVKGFYPSDIAVEWESNGQPENNYKTTPPVLDSDGSFFLYSKLTVDKSRWQQGNVFSCSVMHEALHNHYTQKSLSLSPGK

SEQ ID NO: 49 - protein, 232 aa, Homo sapiens
  source 1..232: note; note (original language) = Human IgG1 Fc region 2
EPKSCDKTHTCPPCPAPEAAGGPSVFLFPPKPKDTLMISRTPEVTCVVVDVSHEDPEVKFNWYVDGVEVHNAKTKPREEQYNSTYRVVSVLTVLHQDWLNGKEYKCKVSNKALPAPIEKTISKAKGQPREPQVYTLPPSRDELTKNQVSLTCLVKGFYPSDIAVEWESNGQPENNYKTTPPVLDSDGSFFLYSKLTVDKSRWQQGNVFSCSVMHEALHNHYTQKSLSLSPGK

SEQ ID NO: 50 - protein, 229 aa, Homo sapiens
  source 1..229: note; note (original language) = Human IgG4 Fc region 1
ESKYGPPCPPCPAPEFEGGPSVFLFPPKPKDTLMISRTPEVTCVVVDVSQEDPEVQFNWYVDGVEVHNAKTKPREEQFNSTYRVVSVLTVLHQDWLNGKEYKCKVSNKGLPSSIEKTISKAKGQPREPQVYTLPPSQEEMTKNQVSLTCLVKGFYPSDIAVEWESNGQPENNYKTTPPVLDSDGSFFLYSRLTVDKSRWQEGNVFSCSVMHEALHNHYTQKSLSLSLGK

SEQ ID NO: 51 - protein, 229 aa, Homo sapiens
  source 1..229: note; note (original language) = Human IgG4 Fc region 2
ESKYGPPCPPCPAPEAAGGPSVFLFPPKPKDTLMISRTPEVTCVVVDVSQEDPEVQFNWYVDGVEVHNAKTKPREEQFNSTYRVVSVLTVLHQDWLNGKEYKCKVSNKGLPSSIEKTISKAKGQPREPQVYTLPPSQEEMTKNQVSLTCLVKGFYPSDIAVEWESNGQPENNYKTTPPVLDSDGSFFLYSRLTVDKSRWQEGNVFSCSVMHEALHNHYTQKSLSLSLGK

SEQ ID NO: 52 - protein, 10 aa, synthetic construct
  source 1..10: note; note (original language) = Linker
GGGGGSGGGG

SEQ ID NO: 53 - protein, 5 aa, synthetic construct
  source 1..5: note; note (original language) = Linker
GGGGS

SEQ ID NO: 54 - protein, 4 aa, synthetic construct
  source 1..4: note; note (original language) = Linker
ASGS

SEQ ID NO: 55 - protein, 4 aa, synthetic construct
  source 1..4: note; note (original language) = Linker
  REGION 1..4: note; note (original language) = (PGPQ)s, wherein s is selected from the group consisting of integers of 1-10 (e.g., 1, 2, 3, 4, 5, or 6)
PGPQ